European Patent Specification EP 3 511 340 B1, published October 2, 2024. Title: Heterodimeric Fc-fused cytokine and pharmaceutical composition comprising the same. Applicant: AJOU UNIVERSITY INDUSTRY-ACADEMIC COOPERATION FOUNDATION. The sequence listing filed with the application follows.

SEQUENCE LISTING (20 sequences)

SEQ ID NO: 1 - protein, 107 aa, Artificial Sequence
  gamma4-EWRVT
GQPREPQVYTLPPSQEEMTENQVSLTCLVKGFYPSDIAVEWESNGQPENNYKTTPPVLDSDGSFFLYSWLTVDKSRWQEGNVFSCSVMHEALHNHYTQKSLSLSLGK

SEQ ID NO: 2 - protein, 107 aa, Artificial Sequence
  gamma4-EWRVT
GQPREPRVYTLPPSQEEMTKNQVSLTCLVKGFYPSDIAVEWESNGQPENNYKTTPPVLVSDGSFTLYSRLTVDKSRWQEGNVFSCSVMHEALHNHYTQKSLSLSLGK

SEQ ID NO: 3 - protein, 107 aa, Artificial Sequence
  gamma4-EWRVTs-s
GQPREPQVCTLPPSQEEMTENQVSLTCLVKGFYPSDIAVEWESNGQPENNYKTTPPVLDSDGSFFLYSWLTVDKSRWQEGNVFSCSVMHEALHNHYTQKSLSLSLGK

SEQ ID NO: 4 - protein, 107 aa, Artificial Sequence
  gamma4-EWRVTs-s
GQPREPRVYTLPPCQEEMTKNQVSLTCLVKGFYPSDIAVEWESNGQPENNYKTTPPVLVSDGSFTLYSRLTVDKSRWQEGNVFSCSVMHEALHNHYTQKSLSLSLGK

SEQ ID NO: 5 - protein, 107 aa, Artificial Sequence
  gamma4-A107
GQPREPQVYTLPPSQEEMTKNQVSLTCLVEGFYPSDIAVEWESNGQPENNYKTTPPVLDSDGSFFLYSWLTVDKSRWQEGNVFSCSVMHEALHNHYTQKSLSLSLGK

SEQ ID NO: 6 - protein, 107 aa, Artificial Sequence
  gamma4-A107
GQPREPQVYTLPPSQENMTKNQVSLTCLVKGFYPSDIAVEWESNGQPENNYKTTPPVLVSDGSFTLYSRLTVDKSRWQEGNVFSCSVMHEALHNHYTQKSLSLSLGK

SEQ ID NO: 7 - protein, 107 aa, Artificial Sequence
  IgG1
GQPREPQVYTLPPSRDELTKNQVSLTCLVKGFYPSDIAVEWESNGQPENNYKTTPPVLDSDGSFFLYSKLTVDKSRWQQGNVFSCSVMHEALHNHYTQKSLSLSPGK

SEQ ID NO: 8 - protein, 107 aa, Artificial Sequence
  gamma1-A107
GQPREPQVYTLPPSRDELTKNQVSLTCLVEGFYPSDIAVEWESNGQPENNYKTTPPVLDSDGSFFLYSWLTVDKSRWQQGNVFSCSVMHEALHNHYTQKSLSLSPGK

SEQ ID NO: 9 - protein, 107 aa, Artificial Sequence
  gamma1-A107
GQPREPQVYTLPPSRDNLTKNQVSLTCLVKGFYPSDIAVEWESNGQPENNYKTTPPVLVSDGSFTLYSKLTVDKSRWQQGNVFSCSVMHEALHNHYTQKSLSLSPGK

SEQ ID NO: 10 - protein, 107 aa, Artificial Sequence
  IgG2
GQPREPQVYTLPPSREEMTKNQVSLTCLVKGFYPSDIAVEWESNGQPENNYKTTPPMLDSDGSFFLYSKLTVDKSRWQQGNVFSCSVMHEALHNHYTQKSLSLSPGK

SEQ ID NO: 11 - protein, 107 aa, Artificial Sequence
  gamma2-A107
GQPREPQVYTLPPSREEMTKNQVSLTCLVEGFYPSDIAVEWESNGQPENNYKTTPPMLDSDGSFFLYSWLTVDKSRWQQGNVFSCSVMHEALHNHYTQKSLSLSPGK

SEQ ID NO: 12 - protein, 107 aa, Artificial Sequence
  gamma2-A107
GQPREPQVYTLPPSRENMTKNQVSLTCLVKGFYPSDIAVEWESNGQPENNYKTTPPMLVSDGSFTLYSKLTVDKSRWQQGNVFSCSVMHEALHNHYTQKSLSLSPGK

SEQ ID NO: 13 - protein, 107 aa, Artificial Sequence
  IgG3
GQPREPQVYTLPPSREEMTKNQVSLTCLVKGFYPSDIAMEWESSGQPENNYKTTPPVLDSDGSFFLYSKLTVDKSRWQQGNIFSCSVMHEALHNHYTQKSLSLSPGK

SEQ ID NO: 14 - protein, 107 aa, Artificial Sequence
  gamma3-A107
GQPREPQVYTLPPSREEMTKNQVSLTCLVEGFYPSDIAMEWESSGQPENNYKTTPPVLDSDGSFFLYSWLTVDKSRWQQGNIFSCSVMHEALHNHYTQKSLSLSPGK

SEQ ID NO: 15 - protein, 107 aa, Artificial Sequence
  gamma3-A107
GQPREPQVYTLPPSRENMTKNQVSLTCLVKGFYPSDIAMEWESSGQPENNYKTTPPVLVSDGSFTLYSKLTVDKSRWQQGNIFSCSVMHEALHNHYTQKSLSLSPGK

SEQ ID NO: 16 - protein, 107 aa, Artificial Sequence
  IgG4
GQPREPQVYTLPPSQEEMTKNQVSLTCLVKGFYPSDIAVEWESNGQPENNYKTTPPVLDSDGSFFLYSRLTVDKSRWQEGNVFSCSVMHEALHNHYTQKSLSLSLGK

SEQ ID NO: 17 - protein, 306 aa, Artificial Sequence
  Mature human IL-12
IWELKKDVYVVELDWYPDAPGEMVVLTCDTPEEDGITWTLDQSSEVLGSGKTLTIRVKEFGDAGQYTCHKGGEVLSHSLLLLHKKEDGIWSTDILKDQKEPKNKTFLRCEAKNYSGRFTCWWLTTISTDLTFSVKSSRGSSDPQGVTCGAATLSAERVRGDNKEYEYSVECQEDSACPAAEESLPIEVMVDAVHKLKYENYTSSFFIRDIIKPDPPKNLQLKPLKNSRQVEVSWEYPDTWSTPHSYFSLTFCVQVQGKSKREKKDRVFTDKTSATVICRKNASISVRAQDRYYSSSWSEWASVPCS

SEQ ID NO: 18 - protein, 197 aa, Artificial Sequence
  Mature human IL-12
RNLPVATPDPGMFPCLHHSQNLLRAVSNMLQKARQTLEFYPCTSEEIDHVDITKDKTSTVEACLPLELTKNESCLNSRETSFITNGSCLASRKTSFMMALCLSSIYEDLKMYQVEFKTMNAKLLMDPKRQIFLDQNMLAVIDELMQALNFNSETVPQKSSLEEPDFYKTKIKLCILLHAFRIRAVTIDRVMSYLNAS

SEQ ID NO: 19 - protein, 313 aa, Artificial Sequence
  Mature mouse IL-12
MWELEKDVYVVEVDWTPDAPGETVNLTCDTPEEDDITWTSDQRHGVIGSGKTLTITVKEFLDAGQYTCHKGGETLSHSHLLLHKKENGIWSTEILKNFKNKTFLKCEAPNYSGRFTCSWLVQRNMDLKFNIKSSSSPPDSRAVTCGMASLSAEKVTLDQRDYEKYSVSCQEDVTCPTAEETLPIELALEARQQNKYENYSTSFFIRDIIKPDPPKNLQMKPLKNSQVEVSWEYPDSWSTPHSYFSLKFFVRIQRKKEKMKETKEGCNQKGAFLVEKTSTEVQCKGGNVCVQAQDRYYNSSCSKWACVPCRVRS

SEQ ID NO: 20 - protein, 193 aa, Artificial Sequence
  Mature mouse IL-12
RVIPVSGPARCLSQSRNLLKTTDDMVKTAREKLKHYSCTAEDIDHEDITRDQTSTLKTCLPLELHKNESCLATRETSSTTRGSCLPPQKTSLMMTLCLGSIYEDLKMYQTEFQAINAALQNHNHQQIILDKGMLVAIDELMQSLNHNGETLRQKPPVGEADPYRVKMKLCILLHAFSTRVVTINRVMGYLSSA